European Patent Application EP 4 141 019 A1, published March 1, 2023. Title: NANO SMALL PEPTIDE FH AND ITS USE IN PREPARATION OF DRUGS FOR TREATING AND PREVENTING FUNDUS VASCULAR DISEASES. Applicant: FUTU Biotech Co., Ltd. Application EP 22192693.4, filed August 29, 2022. The sequence listing filed with the application follows.

SEQUENCE LISTING (2 sequences)

SEQ ID NO: 1 - protein, 12 aa, synthetic construct
FFVLKKQKRPRH

SEQ ID NO: 2 - protein, 12 aa, synthetic construct
FFVLKKNKAAKG